European Patent Specification EP 3 724 238 B1, published March 4, 2026. Title: Heparin and Heparan Sulphate Oligosaccharides. Applicant: Agency for Science, Technology and Reserach. The sequence listing filed with the application follows.

SEQUENCE LISTING (2 sequences)

SEQ ID NO: 1 - protein, 18 aa, Artificial Sequence
  Heparin binding domain of BMP2
QAKHKQRKRLKSSCKRHP

SEQ ID NO: 2 - protein, 17 aa, Artificial Sequence
  Heparin binding domain of BMP2
QAKHKQRKRLKSSCKRH